European Patent Specification EP 3 253 786 B1, published July 1, 2026. Title: OPTIMIZED HUMAN CLOTTING FACTOR VIII GENE EXPRESSION CASSETTES AND THEIR USE. Applicant: The University of North Carolina at Chapel Hill Xiao, Xiao Li, Juan Yuan, Zhenhua. The sequence listing filed with the application follows.

SEQUENCE LISTING (34 sequences)

SEQ ID NO: 1 - DNA, 200 bp, Homo sapiens
ctgtttactctggttaatttttaaaggagggtaaacagtgcctgaaagctgacctttgcccacattcctccggtagacattaacttattaaattgattctgattacaaatctgacctttgcccccatctcacccagtaacaatgcaagagttgatgtcagtctataaaaagcgaagcgcgcggtgggcggggttcgctgc

SEQ ID NO: 2 - DNA, 288 bp, Artificial
  LXP3.3I synthetic promoter sequence
ctgtttactctggttaatttttaaaggagggtaaacagtgcctgaaagctgacctttgcccacattcctccggtagacattaacttattaaattgattctgattacaaatctgacctttgcccccatctcacccagtaacaatgcaagagttgatgtcagtctataaaaagcgaagcgcgcggtgggcggggttcgctgcctgcaggtgagtatctcagggatccagacatggggatatgggaggtgcctctgatcccagggctcactgtgggtctctctgttcacag

SEQ ID NO: 3 - DNA, 4374 bp, Artificial
  Synthetic human B-domain deleted factor FVIII coding sequence
atgcagatcgagctgtctacctgcttcttcctgtgcctgctgcggttctgcttcagcgccaccagacggtactatctgggcgccgtggaactgagctgggactacatgcagagcgacctgggcgagctgcccgtggatgccagattccctccaagagtgcccaagagcttccccttcaacacctccgtggtgtacaagaaaaccctgttcgtggaattcaccgaccacctgttcaatatcgccaagcccagacccccctggatgggcctgctgggacctacaattcaggccgaggtgtacgacaccgtcgtgatcaccctgaagaacatggccagccaccccgtgtctctgcatgccgtgggagtgtcctactggaaggcctctgagggcgccgagtacgacgatcagaccagccagcgcgagaaagaggacgacaaggtgttccctggcggcagccacacctacgtgtggcaggtgctgaaagaaaacggccccatggcctccgaccctctgtgcctgacatacagctacctgagccacgtggacctcgtgaaggacctgaacagcggcctgatcggagccctgctcgtgtgtagagagggcagcctggccaaagagaaaacccagaccctgcacaagttcatcctgctgttcgccgtgttcgacgagggcaagagctggcacagcgagacaaagaacagcctgatgcaggaccgggacgccgcctctgctagagcctggcccaaaatgcacaccgtgaacggctacgtgaacagaagcctgcccggactgatcggctgccaccggaagtctgtgtactggcacgtgatcggcatgggcaccacccctgaggtgcacagcatctttctggaaggacacacctttctcgtgcggaaccaccggcaggccagcctggaaatcagccctatcaccttcctgaccgcccagacactgctgatggacctgggccagtttctgctgttctgccacatcagctcccaccagcacgacggcatggaagcctacgtgaaggtggacagctgccccgaggaaccccagctgcggatgaagaacaacgaggaagccgaggactacgacgacgacctgaccgacagcgagatggacgtggtgcgcttcgacgacgataacagccccagcttcatccagatcagaagcgtggccaagaagcaccccaagacctgggtgcactatatcgccgccgaggaagaggactgggattacgcccctctggtgctggcccccgacgacagaagctacaagagccagtacctgaacaatggcccccagcggatcggccggaagtataagaaagtgcggttcatggcctacaccgacgagacattcaagaccagagaggccatccagcacgagagcggcatcctgggccctctgctgtatggcgaagtgggcgacaccctgctgatcatcttcaagaaccaggccagcagaccctacaacatctaccctcacggcatcaccgacgtgcggcccctgtactctagaaggctgcccaagggcgtgaaacacctgaaggacttccccatcctgcccggcgagattttcaagtacaagtggaccgtgaccgtggaagatggccccaccaagagcgaccccagatgcctgacacggtactacagcagcttcgtgaacatggaacgggacctggcctccggcctgattggcccactgctgatctgctacaaagaaagcgtggaccagcggggcaaccagatcatgagcgacaagcggaacgtgatcctgtttagcgtgttcgatgagaaccggtcctggtatctgaccgagaatatccagcggttcctgcccaaccctgccggcgtgcagctggaagatcctgagttccaggcctccaacatcatgcactccatcaatggctatgtgttcgacagcctgcagctgagcgtgtgcctgcacgaggtggcctactggtacatcctgagcatcggggcccagaccgacttcctgtccgtgttcttctccggctacaccttcaagcacaagatggtgtacgaggataccctgaccctgttcccctttagcggcgaaaccgtgttcatgagcatggaaaaccccggcctgtggatcctgggctgccacaacagcgacttccggaacagaggcatgaccgccctgctgaaggtgtccagctgcgacaagaacaccggcgactactacgaggacagctatgaggacatcagcgcctacctgctgagcaagaacaatgccatcgagcccagaagcttcagccagccccctgtgctgaagcggcaccagagagagatcacccggaccaccctgcagtccgaccaggaagagatcgattacgacgacaccatcagcgtggaaatgaagaaagaagatttcgacatctacgacgaggacgagaaccagagcccccggtcctttcagaaaaagacccggcactacttcattgccgctgtggaacggctgtgggactacggcatgagcagcagccctcacgtgctgagaaacagggcccagagcggcagcgtgccccagttcaagaaagtggtgttccaggaattcacagacggcagctttacccagcctctgtaccgcggcgagctgaacgaacacctgggactgctgggcccctatatccgggccgaagtggaagataacatcatggtcaccttccggaatcaggcctcccggccctacagcttctacagctccctgatcagctacgaagaggaccagagacagggcgctgagccccggaagaacttcgtgaagcccaacgagactaagacctacttttggaaggtgcagcaccacatggcccctacaaaggacgagttcgactgcaaggcctgggcctacttctccgatgtggacctggaaaaggacgtgcactctgggctgatcggccccctgctcgtgtgccacaccaacaccctgaatcccgcccacggcagacaagtgacagtgcaggaattcgccctgttcttcaccatcttcgacgaaacaaagagctggtacttcaccgaaaacatggaaagaaactgccgggctccctgcaacatccagatggaagatcccaccttcaaagagaactaccggttccacgccatcaacggctacatcatggacacactgcccggcctcgtgatggctcaggatcagcggatccggtggtatctgctgtccatgggctccaacgagaacatccacagcatccacttcagcggccacgtgttcaccgtgcggaaaaaagaagagtacaaaatggccctgtacaacctgtaccctggggtgttcgagacagtggaaatgctgcccagcaaggccggcatctggcgggtggaatgtctgatcggcgagcatctgcacgctgggatgagcacactgtttctggtgtacagcaacaagtgccagacacctctgggcatggcctctggccacatccgggactttcagatcacagccagcggccagtatggccagtgggccccaaaactggccagactgcactacagcggcagcatcaacgcctggtccaccaaagagcccttcagctggatcaaggtggacctgctggctcccatgatcatccacggaatcaagacccagggcgccagacagaagttctccagcctgtacatctcccagttcatcatcatgtactccctggacggcaagaagtggcagacctaccggggcaatagcaccggcaccctgatggtgttcttcggcaacgtggactccagcggcattaagcacaacatcttcaacccccccatcattgcccggtacatccggctgcaccccacccactacagcatccggtccaccctgagaatggaactgatgggctgcgacctgaactcctgcagcatgcccctggggatggaaagcaaggccatctccgacgcccagatcaccgcctccagctacttcaccaacatgttcgccacctggtccccatccaaggcccggctgcatctgcagggcagaagcaatgcttggaggccccaagtgaacaaccccaaagaatggctgcaggtggacttccagaaaaccatgaaagtgaccggcgtgaccacccagggcgtgaagtctctgctgacctctatgtacgtgaaagagttcctgatctccagcagccaggacggccaccagtggaccctgtttttccagaacggcaaagtgaaagtgtttcaggggaaccaggacagcttcacccccgtcgtgaatagcctggaccctccactgctgaccagatacctgcggatccaccctcagagttgggtgcaccagattgctctgcggatggaagtgctgggatgcgaggcccaggacctgtactgataa

SEQ ID NO: 4 - DNA, 5045 bp, Artificial
  Recombinant AAV vector sequence
ttggccactccctctctgcgcgctcgctcgctcactgaggccgggcgaccaaaggtcgcccgacgcccgggctttgcccgggcggcctcagtgagcgagcgagcgcgcagagagggagtggccaactccatcactaggggttcctagatctacgcgtctgtttactctggttaatttttaaaggagggtaaacagtgcctgaaagctgacctttgcccacattcctccggtagacattaacttattaaattgattctgattacaaatctgacctttgcccccatctcacccagtaacaatgcaagagttgatgtcagtctataaaaagcgaagcgcgcggtgggcggggttcgctgcctgcaggtgagtatctcagggatccagacatggggatatgggaggtgcctctgatcccagggctcactgtgggtctctctgttcacagcctgctagcgccaccatgcagatcgagctgtctacctgcttcttcctgtgcctgctgcggttctgcttcagcgccaccagacggtactatctgggcgccgtggaactgagctgggactacatgcagagcgacctgggcgagctgcccgtggatgccagattccctccaagagtgcccaagagcttccccttcaacacctccgtggtgtacaagaaaaccctgttcgtggaattcaccgaccacctgttcaatatcgccaagcccagacccccctggatgggcctgctgggacctacaattcaggccgaggtgtacgacaccgtcgtgatcaccctgaagaacatggccagccaccccgtgtctctgcatgccgtgggagtgtcctactggaaggcctctgagggcgccgagtacgacgatcagaccagccagcgcgagaaagaggacgacaaggtgttccctggcggcagccacacctacgtgtggcaggtgctgaaagaaaacggccccatggcctccgaccctctgtgcctgacatacagctacctgagccacgtggacctcgtgaaggacctgaacagcggcctgatcggagccctgctcgtgtgtagagagggcagcctggccaaagagaaaacccagaccctgcacaagttcatcctgctgttcgccgtgttcgacgagggcaagagctggcacagcgagacaaagaacagcctgatgcaggaccgggacgccgcctctgctagagcctggcccaaaatgcacaccgtgaacggctacgtgaacagaagcctgcccggactgatcggctgccaccggaagtctgtgtactggcacgtgatcggcatgggcaccacccctgaggtgcacagcatctttctggaaggacacacctttctcgtgcggaaccaccggcaggccagcctggaaatcagccctatcaccttcctgaccgcccagacactgctgatggacctgggccagtttctgctgttctgccacatcagctcccaccagcacgacggcatggaagcctacgtgaaggtggacagctgccccgaggaaccccagctgcggatgaagaacaacgaggaagccgaggactacgacgacgacctgaccgacagcgagatggacgtggtgcgcttcgacgacgataacagccccagcttcatccagatcagaagcgtggccaagaagcaccccaagacctgggtgcactatatcgccgccgaggaagaggactgggattacgcccctctggtgctggcccccgacgacagaagctacaagagccagtacctgaacaatggcccccagcggatcggccggaagtataagaaagtgcggttcatggcctacaccgacgagacattcaagaccagagaggccatccagcacgagagcggcatcctgggccctctgctgtatggcgaagtgggcgacaccctgctgatcatcttcaagaaccaggccagcagaccctacaacatctaccctcacggcatcaccgacgtgcggcccctgtactctagaaggctgcccaagggcgtgaaacacctgaaggacttccccatcctgcccggcgagattttcaagtacaagtggaccgtgaccgtggaagatggccccaccaagagcgaccccagatgcctgacacggtactacagcagcttcgtgaacatggaacgggacctggcctccggcctgattggcccactgctgatctgctacaaagaaagcgtggaccagcggggcaaccagatcatgagcgacaagcggaacgtgatcctgtttagcgtgttcgatgagaaccggtcctggtatctgaccgagaatatccagcggttcctgcccaaccctgccggcgtgcagctggaagatcctgagttccaggcctccaacatcatgcactccatcaatggctatgtgttcgacagcctgcagctgagcgtgtgcctgcacgaggtggcctactggtacatcctgagcatcggggcccagaccgacttcctgtccgtgttcttctccggctacaccttcaagcacaagatggtgtacgaggataccctgaccctgttcccctttagcggcgaaaccgtgttcatgagcatggaaaaccccggcctgtggatcctgggctgccacaacagcgacttccggaacagaggcatgaccgccctgctgaaggtgtccagctgcgacaagaacaccggcgactactacgaggacagctatgaggacatcagcgcctacctgctgagcaagaacaatgccatcgagcccagaagcttcagccagccccctgtgctgaagcggcaccagagagagatcacccggaccaccctgcagtccgaccaggaagagatcgattacgacgacaccatcagcgtggaaatgaagaaagaagatttcgacatctacgacgaggacgagaaccagagcccccggtcctttcagaaaaagacccggcactacttcattgccgctgtggaacggctgtgggactacggcatgagcagcagccctcacgtgctgagaaacagggcccagagcggcagcgtgccccagttcaagaaagtggtgttccaggaattcacagacggcagctttacccagcctctgtaccgcggcgagctgaacgaacacctgggactgctgggcccctatatccgggccgaagtggaagataacatcatggtcaccttccggaatcaggcctcccggccctacagcttctacagctccctgatcagctacgaagaggaccagagacagggcgctgagccccggaagaacttcgtgaagcccaacgagactaagacctacttttggaaggtgcagcaccacatggcccctacaaaggacgagttcgactgcaaggcctgggcctacttctccgatgtggacctggaaaaggacgtgcactctgggctgatcggccccctgctcgtgtgccacaccaacaccctgaatcccgcccacggcagacaagtgacagtgcaggaattcgccctgttcttcaccatcttcgacgaaacaaagagctggtacttcaccgaaaacatggaaagaaactgccgggctccctgcaacatccagatggaagatcccaccttcaaagagaactaccggttccacgccatcaacggctacatcatggacacactgcccggcctcgtgatggctcaggatcagcggatccggtggtatctgctgtccatgggctccaacgagaacatccacagcatccacttcagcggccacgtgttcaccgtgcggaaaaaagaagagtacaaaatggccctgtacaacctgtaccctggggtgttcgagacagtggaaatgctgcccagcaaggccggcatctggcgggtggaatgtctgatcggcgagcatctgcacgctgggatgagcacactgtttctggtgtacagcaacaagtgccagacacctctgggcatggcctctggccacatccgggactttcagatcacagccagcggccagtatggccagtgggccccaaaactggccagactgcactacagcggcagcatcaacgcctggtccaccaaagagcccttcagctggatcaaggtggacctgctggctcccatgatcatccacggaatcaagacccagggcgccagacagaagttctccagcctgtacatctcccagttcatcatcatgtactccctggacggcaagaagtggcagacctaccggggcaatagcaccggcaccctgatggtgttcttcggcaacgtggactccagcggcattaagcacaacatcttcaacccccccatcattgcccggtacatccggctgcaccccacccactacagcatccggtccaccctgagaatggaactgatgggctgcgacctgaactcctgcagcatgcccctggggatggaaagcaaggccatctccgacgcccagatcaccgcctccagctacttcaccaacatgttcgccacctggtccccatccaaggcccggctgcatctgcagggcagaagcaatgcttggaggccccaagtgaacaaccccaaagaatggctgcaggtggacttccagaaaaccatgaaagtgaccggcgtgaccacccagggcgtgaagtctctgctgacctctatgtacgtgaaagagttcctgatctccagcagccaggacggccaccagtggaccctgtttttccagaacggcaaagtgaaagtgtttcaggggaaccaggacagcttcacccccgtcgtgaatagcctggaccctccactgctgaccagatacctgcggatccaccctcagagttgggtgcaccagattgctctgcggatggaagtgctgggatgcgaggcccaggacctgtactgataagtcgacaggcctaataaagagctcagatgcatcgatcagagtgtgttggttttttgtgtgagatctaggaacccctagtgatggagttggccactccctctctgcgcgctcgctcgctcactgaggccgcccgggcaaagcccgggcgtcgggcgacctttggtcgcccggcctcagtgagcgagcgagcgcgcagagagggagtggccaa

SEQ ID NO: 5 - protein, 2333 aa, Homo sapiens
ATRRYYLGAVELSWDYMQSDLGELPVDARFPPRVPKSFPFNTSVVYKKTLFVEFTVHLFNIAKPRPPWMGLLGPTIQAEVYDTVVITLKNMASHPVSLHAVGVSYWKASEGAEYDDQTSQREKEDDKVFPGGSHTYVWQVLKENGPMASDPLCLTYSYLSHVDLVKDLNSGLIGALLVCREGSLAKEKTQTLHKFILLFAVFDEGKSWHSETKNSLMQDRDAASARAWPKMHTVNGYVNRSLPGLIGCHRKSVYWHVIGMGTTPEVHSIFLEGHTFLVRNHRQASLEISPITFLTAQTLLMDLGQFLLFCHISSHQHDGMEAYVKVDSCPEEPQLRMKNNEEAEDYDDDLTDSEMDVVRFDDDNSPSFIQIRSVAKKHPKTWVHYIAAEEEDWDYAPLVLAPDDRSYKSQYLNNGPQRIGRKYKKVRFMAYTDETFKTREAIQHESGILGPLLYGEVGDTLLIIFKNQASRPYNIYPHGITDVRPLYSRRLPKGVKHLKDFPILPGEIFKYKWTVTVEDGPTKSDPRCLTRYYSSFVNMERDLASGLIGPLLICYKESVDQRGNQIMSDKRNVILFSVFDENRSWYLTENIQRFLPNPAGVQLEDPEFQASNIMHSINGYVFDSLQLSVCLHEVAYWYILSIGAQTDFLSVFFSGYTFKHKMVYEDTLTLFPFSGETVFMSMENPGLWILGCHNSDFRNRGMTALLKVSSCDKNTGDYYEDSYEDISAYLLSKNNAIEPRSFSQNSRHPSTRQKQFNATTIPENDIEKTDPWFAHRTPMPKIQNVSSSDLLMLLRQSPTPHGLSLSDLQEAKYETFSDDPSPGAIDSNNSLSEMTHFRPQLHHSGDMVFTPESGLQLRLNEKLGTTAATELKKLDFKVSSTSNNLISTIPSDNLAAGTDNTSSLGPPSMPVHYDSQLDTTLFGKKSSPLTESGGPLSLSEENNDSKLLESGLMNSQESSWGKNVSSTESGRLFKGKRAHGPALLTKDNALFKVSISLLKTNKTSNNSATNRKTHIDGPSLLIENSPSVWQNILESDTEFKKVTPLIHDRMLMDKNATALRLNHMSNKTTSSKNMEMVQQKKEGPIPPDAQNPDMSFFKMLFLPESARWIQRTHGKNSLNSGQGPSPKQLVSLGPEKSVEGQNFLSEKNKVVVGKGEFTKDVGLKEMVFPSSRNLFLTNLDNLHENNTHNQEKKIQEEIEKKETLIQENVVLPQIHTVTGTKNFMKNLFLLSTRQNVEGSYEGAYAPVLQDFRSLNDSTNRTKKHTAHFSKKGEEENLEGLGNQTKQIVEKYACTTRISPNTSQQNFVTQRSKRALKQFRLPLEETELEKRIIVDDTSTQWSKNMKHLTPSTLTQIDYNEKEKGAITQSPLSDCLTRSHSIPQANRSPLPIAKVSSFPSIRPIYLTRVLFQDNSSHLPAASYRKKDSGVQESSHFLQGAKKNNLSLAILTLEMTGDQREVGSLGTSATNSVTYKKVENTVLPKPDLPKTSGKVELLPKVHIYQKDLFPTETSNGSPGHLDLVEGSLLQGTEGAIKWNEANRPGKVPFLRVATESSAKTPSKLLDPLAWDNHYGTQIPKEEWKSQEKSPEKTAFKKKDTILSLNACESNHAIAAINEGQNKPEIEVTWAKQGRTERLCSQNPPVLKRHQREITRTTLQSDQEEIDYDDTISVEMKKEDFDIYDEDENQSPRSFQKKTRHYFIAAVERLWDYGMSSSPHVLRNRAQSGSVPQFKKVVFQEFTDGSFTQPLYRGELNEHLGLLGPYIRAEVEDNIMVTFRNQASRPYSFYSSLISYEEDQRQGAEPRKNFVKPNETKTYFWKVQHHMAPTKDEFBDCKAWAYFSDVDLEKDVHSGLIGPLLVCHTNTLNPAHGRQVTVQEFALFFTIFDETKSWYFTENMERNCRAPCNIQMEDPTFKENYRFHAINGYIMDTLPGLVMAQDQRIRWYLLSMGSNENIHSIHFSGHVFTVRKKEEYKMALYNLYPGVFETVEMLPSKAGIWRVECLIGEHLHAGMSTLFLVYSNKCQTPLGMASGHIRDFQITASGQYGQWAPKLARLHYSGSINAWSTKEPFSWIKVDLLAPMIIHGIKTQGARQKFSSLYISQFIIMYSLDGKKWQTYRGNSTGTLMVFFGNVDSSGIKHNIFNPPIIARYIRLHPTHYSIRSTLRMELMGCDLNSCSMPLGMESKAISDAQITASSYFTNMFATWSPSKARLHLQGRSNAWRPQVNNPKEWLQVDFQKTMKVTGVTTQGVKSLLTSMYVKEFLISSSQDGHQWTLFFQNGKVKVFQGNQDSFTPVVNSLDPPLLTRYLRIHPQSWVHQIALRMEVLGCEAQDLY

SEQ ID NO: 6 - protein, 8 aa, Artificial
  Factor VIII consensus insert sequence
  MISC_FEATURE (1)..(2): Xaa can be S or T
  MISC_FEATURE (7)..(7): Xaa can be S or T
XXYVNRXL

SEQ ID NO: 7 - protein, 8 aa, Artificial
  Factor VIII insert sequence
TTYVNRSL

SEQ ID NO: 8 - protein, 8 aa, Artificial
  Factor VIII insert sequence
TTYVNRTL

SEQ ID NO: 9 - protein, 8 aa, Artificial
  Factor VIII insert sequence
TSYVNRSL

SEQ ID NO: 10 - protein, 8 aa, Artificial
  Factor VIII insert sequence
TSYVNRTL

SEQ ID NO: 11 - protein, 8 aa, Artificial
  Factor VIII insert sequence
STYVNRSL

SEQ ID NO: 12 - protein, 8 aa, Artificial
  Factor VIII insert sequence
STYVNRTL

SEQ ID NO: 13 - protein, 8 aa, Artificial
  Factor VIII insert sequence
SSYVNRSL

SEQ ID NO: 14 - protein, 8 aa, Artificial
  Factor VIII insert sequence
SSYVNRTL

SEQ ID NO: 15 - protein, 5 aa, Artificial
  Factor VIII consensus insert sequence
  MISC_FEATURE (1)..(2): Xaa can be S or T
  MISC_FEATURE (5)..(5): Xaa can be S or T
XXNNX

SEQ ID NO: 16 - protein, 5 aa, Artificial
  Factor VIII insert sequence
TTNNS

SEQ ID NO: 17 - protein, 5 aa, Artificial
  Factor VIII insert sequence
TTNNT

SEQ ID NO: 18 - protein, 5 aa, Artificial
  Factor VIII insert sequence
TSNNS

SEQ ID NO: 19 - protein, 5 aa, Artificial
  Factor VIII insert sequence
TSNNT

SEQ ID NO: 20 - protein, 5 aa, Artificial
  Factor VIII insert sequence
STNNS

SEQ ID NO: 21 - protein, 5 aa, Artificial
  Factor VIII insert sequence
STNNT

SEQ ID NO: 22 - protein, 5 aa, Artificial
  Factor VIII insert sequence
SSNNS

SEQ ID NO: 23 - protein, 5 aa, Artificial
  Factor VIII insert sequence
SSNNT

SEQ ID NO: 24 - protein, 7 aa, Artificial
  O-linked glycosylation site consensus sequence
  misc_feature (2)..(3): Xaa can be any naturally occurring amino acid
  MISC_FEATURE (6)..(6): Xaa can be S or T
CXXGGXC

SEQ ID NO: 25 - protein, 5 aa, Artificial
  O-linked glycosylation site sequence
  MISC_FEATURE (4)..(4): Xaa can be D or E
NSTXA

SEQ ID NO: 26 - protein, 5 aa, Artificial
  O-linked glycosylation site sequence
NITQS

SEQ ID NO: 27 - protein, 5 aa, Artificial
  O-linked glycosylation site sequence
QSTQS

SEQ ID NO: 28 - protein, 5 aa, Artificial
  O-linked glycosylation site sequence
  MISC_FEATURE (1)..(1): Xaa can be D or E
  MISC_FEATURE (4)..(4): Xaa can be R or K
XFTXV

SEQ ID NO: 29 - protein, 4 aa, Artificial
  O-linked glycosylation site sequence
  MISC_FEATURE (2)..(2): Xaa can be D or E
CXSN

SEQ ID NO: 30 - protein, 5 aa, Artificial
  O-linked glycosylation site sequence
  MISC_FEATURE (5)..(5): Xaa can be R or K
GGSCX

SEQ ID NO: 31 - protein, 30 aa, Artificial
  B domain deleted Factor VIII sequence
LSKNNAIEPRSFSQNPPVLKRHQREITRTT

SEQ ID NO: 32 - protein, 30 aa, Artificial
  Mutated B domain deleted Factor VIII sequence
LSKNNTTEPRSFSQNPPVLKRHQREITRTT

SEQ ID NO: 33 - protein, 31 aa, Artificial
  Mutated B domain deleted Factor VIII sequence
LSKNNTTYVNRSLSQNPPVLKRHQREITRTT

SEQ ID NO: 34 - protein, 28 aa, Artificial
  Mutated B domain deleted Factor VIII sequence
LSKNNTTNNTSQNPPVLKRHQREITRTT